European Patent Specification EP 3 724 223 B1, published June 3, 2026. Title: NEUTRALIZING ANTIBODIES TO EBOLA VIRUS GLYCOPROTEIN. Applicant: THE UNITED STATES OF AMERICA, AS REPRESENTED BY THE SECRETARY, DEPARTMENT OF HEALTH AND HUMAN SERVICES. The sequence listing filed with the application follows.

SEQUENCE LISTING (31 sequences)

SEQ ID NO: 1 - protein, 125 aa, Artificial Sequence
  Synthetic polypeptide
QVQLQESGPGLVKPSETLSLTCVVSGGILSSFYWNWIRQPPGKGLEWIGNIYYSGSPNYNASFQSRVAISVDTSKNQISLNLKSVTAADTAMYYCVRASRAYLWGSYRPTALDLWGQGSLVTVSS

SEQ ID NO: 2 - protein, 105 aa, Artificial Sequence
  Synthetic polypeptide
SYELTQPPSVSVSPGQTATITCSGDKLGDKYTSWFQQRPGQSPLLVIYQDNKRPSGLPARFSGSNSGNTATLTISGTQAMDEADYLCQVWDSGAVFGGGTKLTVL

SEQ ID NO: 3 - protein, 125 aa, Artificial Sequence
  Synthetic polypeptide
QVQLQESGPGLVKPSETLSLTCVVSGGILSSFYWNWIRQPPGKGLEWIGNIYYSGSPNYNPSFQSRVAISVDTSKNQISLNLKSVTAADTAMYYCVRASRAYLWGSYRPTALDLWGQGSLVTVSS

SEQ ID NO: 4 - protein, 455 aa, Artificial Sequence
  Synthetic polypeptide
QVQLQESGPGLVKPSETLSLTCVVSGGILSSFYWNWIRQPPGKGLEWIGNIYYSGSPNYNASFQSRVAISVDTSKNQISLNLKSVTAADTAMYYCVRASRAYLWGSYRPTALDLWGQGSLVTVSSASTKGPSVFPLAPSSKSTSGGTAALGCLVKDYFPEPVTVSWNSGALTSGVHTFPAVLQSSGLYSLSSVVTVPSSSLGTQTYICNVNHKPSNTKVDKKVEPKSCDKTHTCPPCPAPELLGGPSVFLFPPKPKDTLMISRTPEVTCVVVDVSHEDPEVKFNWYVDGVEVHNAKTKPREEQYNSTYRVVSVLTVLHQDWLNGKEYKCKVSNKALPAPIEKTISKAKGQPREPQVYTLPPSRDELTKNQVSLTCLVKGFYPSDIAVEWESNGQPENNYKTTPPVLDSDGSFFLYSKLTVDKSRWQQGNVFSCSVMHEALHNHYTQKSLSLSPGK

SEQ ID NO: 5 - protein, 211 aa, Artificial Sequence
  Synthetic polypeptide
SYELTQPPSVSVSPGQTATITCSGDKLGDKYTSWFQQRPGQSPLLVIYQDNKRPSGLPARFSGSNSGNTATLTISGTQAMDEADYLCQVWDSGAVFGGGTKLTVLGQPKAAPSVTLFPPSSEELQANKATLVCLISDFYPGAVTVAWKADSSPVKAGVETTTPSKQSNNKYAASSYLSLTPEQWKSHRSYSCQVTHEGSTVEKTVAPTECS

SEQ ID NO: 6 - protein, 455 aa, Artificial Sequence
  Synthetic polypeptide
QVQLQESGPGLVKPSETLSLTCVVSGGILSSFYWNWIRQPPGKGLEWIGNIYYSGSPNYNPSFQSRVAISVDTSKNQISLNLKSVTAADTAMYYCVRASRAYLWGSYRPTALDLWGQGSLVTVSSASTKGPSVFPLAPSSKSTSGGTAALGCLVKDYFPEPVTVSWNSGALTSGVHTFPAVLQSSGLYSLSSVVTVPSSSLGTQTYICNVNHKPSNTKVDKKVEPKSCDKTHTCPPCPAPELLGGPSVFLFPPKPKDTLMISRTPEVTCVVVDVSHEDPEVKFNWYVDGVEVHNAKTKPREEQYNSTYRVVSVLTVLHQDWLNGKEYKCKVSNKALPAPIEKTISKAKGQPREPQVYTLPPSRDELTKNQVSLTCLVKGFYPSDIAVEWESNGQPENNYKTTPPVLDSDGSFFLYSKLTVDKSRWQQGNVFSCSVMHEALHNHYTQKSLSLSPGK

SEQ ID NO: 7 - protein, 8 aa, Artificial Sequence
  Synthetic polypeptide
GGILSSFY

SEQ ID NO: 8 - protein, 7 aa, Artificial Sequence
  Synthetic polypeptide
IYYSGSP

SEQ ID NO: 9 - protein, 19 aa, Artificial Sequence
  Synthetic polypeptide
VRASRAYLWGSYRPTALDL

SEQ ID NO: 10 - protein, 6 aa, Artificial Sequence
  Synthetic polypeptide
KLGDKY

SEQ ID NO: 11 - protein, 3 aa, Artificial Sequence
  Synthetic polypeptide
QDN

SEQ ID NO: 12 - protein, 8 aa, Artificial Sequence
  Synthetic polypeptide
QVWDSGAV

SEQ ID NO: 13 - DNA, 432 bp, Artificial Sequence
  Synthetic polynucleotide
atgggatggtcatgtatcatcctttttctagtagcaactgcaaccggtgtacattctcaggtgcagctgcaggagtcgggaccaggactggtgaagccttcggagaccctgtccctcacctgcgttgtctctggtggcatcctcagtagtttttactggaactggatccggcagcccccaggaaagggactggagtggattggaaacatctattacagtgggagccccaactataatgcctccttccagagtcgagtcgccatttcggtggacacgtccaagaaccagatctccctgaacctcaagtctgtgaccgctgcggacacggccatgtattactgtgtgagagcctcccgcgcttacctttgggggagttatcgtccaacggctcttgacctctggggccagggatccctggtcaccgtctcctca

SEQ ID NO: 14 - DNA, 372 bp, Artificial Sequence
  Synthetic polynucleotide
atgggatggtcatgtatcatcctttttctagtagcaactgcaaccggtgtccatgcttcctatgagctgactcagccaccctcagtgtccgtgtccccaggacagacagccaccatcacgtgctctggagataaattgggtgataaatatacttcctggttccagcagaggccaggccagtcccctctactggtcatctatcaggataataagcggccctcagggctccctgcgcgattttctggctccaactctgggaacacagccactctgaccatcagcggcacccaggctatggatgaggctgactatttgtgtcaggtgtgggacagcggtgcggtgttcggcggagggaccaagctgaccgtccta

SEQ ID NO: 15 - DNA, 432 bp, Artificial Sequence
  Synthetic polynucleotide
atgggatggtcatgtatcatcctttttctagtagcaactgcaaccggtgtacattctcaggtgcagctgcaggagtcgggaccaggactggtgaagccttcggagaccctgtccctcacctgcgttgtctctggtggcatcctcagtagtttttactggaactggatccggcagcccccaggaaagggactggagtggattggaaacatctattacagtgggagccccaactataatccctccttccagagtcgagtcgccatttcggtggacacgtccaagaaccagatctccctgaacctcaagtctgtgaccgctgcggacacggccatgtattactgtgtgagagcctcccgcgcttacctttgggggagttatcgtccaacggctcttgacctctggggccagggatccctggtcaccgtctcctca

SEQ ID NO: 16 - DNA, 1425 bp, Artificial Sequence
  Synthetic nucleic acid
atgggatggtcatgtatcatcctttttctagtagcaactgcaaccggtgtacattctcaggtgcagctgcaggagtcgggaccaggactggtgaagccttcggagaccctgtccctcacctgcgttgtctctggtggcatcctcagtagtttttactggaactggatccggcagcccccaggaaagggactggagtggattggaaacatctattacagtgggagccccaactataatgcctccttccagagtcgagtcgccatttcggtggacacgtccaagaaccagatctccctgaacctcaagtctgtgaccgctgcggacacggccatgtattactgtgtgagagcctcccgcgcttacctttgggggagttatcgtccaacggctcttgacctctggggccagggatccctggtcaccgtctcctcagcgtcgaccaagggcccatcggtcttccccctggcaccctcctccaagagcacctctgggggcacagcggccctgggctgcctggtcaaggactacttccccgaacccgtgacggtgtcgtggaactcaggcgccctgaccagcggcgtgcacaccttcccggctgtcctacagtcctcaggactctactccctcagcagcgtggtgaccgtgccctccagcagcttgggcacccagacctacatctgcaacgtgaatcacaagcccagcaacaccaaggtggacaagaaagttgagcccaaatcttgtgacaaaactcacacatgcccaccgtgcccagcacctgaactcctggggggaccgtcagtcttcctcttccccccaaaacccaaggacaccctcatgatctcccggacccctgaggtcacatgcgtggtggtggacgtgagccacgaagaccctgaggtcaagttcaactggtacgtggacggcgtggaggtgcataatgccaagacaaagccgcgggaggagcagtacaacagcacgtaccgtgtggtcagcgtcctcaccgtcctgcaccaggactggctgaatggcaaggagtacaagtgcaaggtctccaacaaagccctcccagcccccatcgagaaaaccatctccaaagccaaagggcagccccgagaaccacaggtgtacaccctgcccccatcccgggatgagctgaccaagaaccaggtcagcctgacctgcctggtcaaaggcttctatcccagcgacatcgccgtggagtgggagagcaatgggcagccggagaacaactacaagaccacgcctcccgtgctggactccgacggctccttcttcctctacagcaagctcaccgtggacaagagcaggtggcagcaggggaacgtcttctcatgctccgtgatgcatgaggctctgcacaaccactacacgcagaagagcctctccctgtctccgggtaaatga

SEQ ID NO: 17 - DNA, 693 bp, Artificial Sequence
  Synthetic nucleic acid
atgggatggtcatgtatcatcctttttctagtagcaactgcaaccggtgtccatgcttcctatgagctgactcagccaccctcagtgtccgtgtccccaggacagacagccaccatcacgtgctctggagataaattgggtgataaatatacttcctggttccagcagaggccaggccagtcccctctactggtcatctatcaggataataagcggccctcagggctccctgcgcgattttctggctccaactctgggaacacagccactctgaccatcagcggcacccaggctatggatgaggctgactatttgtgtcaggtgtgggacagcggtgcggtgttcggcggagggaccaagctgaccgtcctaggtcagcccaaggctgccccctcggtcactctgttcccaccctcgagtgaggagcttcaagccaacaaggccacactggtgtgtctcataagtgacttctacccgggagccgtgacagtggcctggaaggcagatagcagccccgtcaaggcgggagtggagaccaccacaccctccaaacaaagcaacaacaagtacgcggccagcagctacctgagcctgacgcctgagcagtggaagtcccacagaagctacagctgccaggtcacgcatgaagggagcaccgtggagaagacagtggcccctacagaatgttcatag

SEQ ID NO: 18 - DNA, 1425 bp, Artificial Sequence
  Synthetic nucleic acid
atgggatggtcatgtatcatcctttttctagtagcaactgcaaccggtgtacattctcaggtgcagctgcaggagtcgggaccaggactggtgaagccttcggagaccctgtccctcacctgcgttgtctctggtggcatcctcagtagtttttactggaactggatccggcagcccccaggaaagggactggagtggattggaaacatctattacagtgggagccccaactataatccctccttccagagtcgagtcgccatttcggtggacacgtccaagaaccagatctccctgaacctcaagtctgtgaccgctgcggacacggccatgtattactgtgtgagagcctcccgcgcttacctttgggggagttatcgtccaacggctcttgacctctggggccagggatccctggtcaccgtctcctcagcgtcgaccaagggcccatcggtcttccccctggcaccctcctccaagagcacctctgggggcacagcggccctgggctgcctggtcaaggactacttccccgaacccgtgacggtgtcgtggaactcaggcgccctgaccagcggcgtgcacaccttcccggctgtcctacagtcctcaggactctactccctcagcagcgtggtgaccgtgccctccagcagcttgggcacccagacctacatctgcaacgtgaatcacaagcccagcaacaccaaggtggacaagaaagttgagcccaaatcttgtgacaaaactcacacatgcccaccgtgcccagcacctgaactcctggggggaccgtcagtcttcctcttccccccaaaacccaaggacaccctcatgatctcccggacccctgaggtcacatgcgtggtggtggacgtgagccacgaagaccctgaggtcaagttcaactggtacgtggacggcgtggaggtgcataatgccaagacaaagccgcgggaggagcagtacaacagcacgtaccgtgtggtcagcgtcctcaccgtcctgcaccaggactggctgaatggcaaggagtacaagtgcaaggtctccaacaaagccctcccagcccccatcgagaaaaccatctccaaagccaaagggcagccccgagaaccacaggtgtacaccctgcccccatcccgggatgagctgaccaagaaccaggtcagcctgacctgcctggtcaaaggcttctatcccagcgacatcgccgtggagtgggagagcaatgggcagccggagaacaactacaagaccacgcctcccgtgctggactccgacggctccttcttcctctacagcaagctcaccgtggacaagagcaggtggcagcaggggaacgtcttctcatgctccgtgatgcatgaggctctgcacaaccactacacgcagaagagcctctccctgtctccgggtaaatga

SEQ ID NO: 19 - protein, 19 aa, Artificial Sequence
  Synthetic polypeptide
MGWSCIILFLVATATGVHS

SEQ ID NO: 20 - protein, 19 aa, Artificial Sequence
  Synthetic polypeptide
MGWSCIILFLVATATGVHA

SEQ ID NO: 21 - protein, 119 aa, Artificial Sequence [sequence omitted]

SEQ ID NO: 22 - protein, 107 aa, Artificial Sequence [sequence omitted]

SEQ ID NO: 23 - protein, 125 aa, Artificial Sequence
  Synthetic polypeptide
QVQLQESGPGLVKPSDTLSLTCTVSGGSLSSFYWSWIRQPPGKGLEWIGYIYYSGSPNYSPSLESRVTMSVDTTRNQISLKLDSVTAADTAVYYCVRASRSYYWGSYRPTAFDSWGQGTLVTVSS

SEQ ID NO: 24 - protein, 105 aa, Artificial Sequence
  Synthetic polypeptide
SYELTQPLSVSVSPGQTAIFTCSGDNLGDKYVCWFQQRPGQSPMLLIYQDNKRPSGIPERFSGSNSGNTATLTISGTQSTDEADYYCQTWDSTVVFGGGTKLTVL

SEQ ID NO: 25 - protein, 676 aa, Bundibugyo ebolavirus
MVTSGILQLPRERFRKTSFFVWVIILFHKVFPIPLGVVHNNTLQVSDIDKLVCRDKLSSTSQLKSVGLNLEGNGVATDVPTATKRWGFRAGVPPKVVNYEAGEWAENCYNLDIKKADGSECLPEAPEGVRGFPRCRYVHKVSGTGPCPEGYAFHKEGAFFLYDRLASTIIYRSTTFSEGVVAFLILPETKKDFFQSPPLHEPANMTTDPSSYYHTVTLNYVADNFGTNMTNFLFQVDHLTYVQLEPRFTPQFLVQLNETIYTNGRRSNTTGTLIWKVNPTVDTGVGEWAFWENKKNFTKTLSSEELSVIFVPRAQDPGSNQKTKVTPTSFANNQTSKNHEDLVPEDPASVVQVRDLQRENTVPTPPPDTVPTTLIPDTMEEQTTSHYEPPNISRNHQERNNTAHPETLANNPPDNTTPSTPPQDGERTSSHTTPSPRPVPTSTIHPTTRETHIPTTMTTSHDTDSNRPNPIDISESTEPGPLTNTTRGAANLLTGSRRTRREITLRTQAKCNPNLHYWTTQDEGAAIGLAWIPYFGPAAEGIYTEGIMHNQNGLICGLRQLANETTQALQLFLRATTELRTFSILNRKAIDFLLQRWGGTCHILGPDCCIEPHDWTKNITDKIDQIIHDFIDKPLPDQTDNDNWWTGWRQWVPAGIGITGVIIAVIALLCICKFLL

SEQ ID NO: 26 - protein, 676 aa, Sudan ebolavirus
MEGLSLLQLPRDKFRKSSFFVWVIILFQKAFSMPLGVVTNSTLEVTEIDQLVCKDHLASTDQLKSVGLNLEGSGVSTDIPSATKRWGFRSGVPPKVFSYEAGEWAENCYNLEIKKPDGSECLPPPPDGVRGFPRCRYVHKAQGTGPCPGDYAFHKDGAFFLYDRLASTVIYRGVNFAEGVIAFLILAKPKETFLQSPPIREAVNYTENTSSYYATSYLEYEIENFGAQHSTTLFKINNNTFVLLDRPHTPQFLFQLNDTIHLHQQLSNTTGKLIWTLDANINADIGEWAFWENKKNLSEQLRGEELSFETLSLNETEDDDATSSRTTKGRISDRATRKYSDLVPKDSPGMVSLHVPEGETTLPSQNSTEGRRVDVNTQETITETTATIIGTNGNNMQISTIGTGLSSSQILSSSPTMAPSPETQTSTTYTPKLPVMTTEESTTPPRNSPGSTTEAPTLTTPENITTAVKTVLPQESTSNGLITSTVTGILGSLGLRKRSRRQVNTRATGKCNPNLHYWTAQEQHNAAGIAWIPYFGPGAEGIYTEGLMHNQNALVCGLRQLANETTQALQLFLRATTELRTYTILNRKAIDFLLRRWGGTCRILGPDCCIEPHDWTKNITDKINQIIHDFIDNPLPNQDNDDNWWTGWRQWIPAGIGITGIIIAIIALLCVCKLLC

SEQ ID NO: 27 - protein, 676 aa, Zaire ebolavirus
MGVTGILQLPRDRFKKTSFFLWVIILFQRTFSIPLGVIHNSTLQVSDVDKLVCRDKLSSTNQLRSVGLNLEGNGVATDVPSATKRWGFRSGVPPKVVNYEAGEWAENCYNLEIKKPDGSECLPAAPDGIRGFPRCRYVHKVSGTGPCAGDFAFHKEGAFFLYDRLASTVIYRGTTFAEGVVAFLILPQAKKDFFSSHPLREPVNATEDPSSGYYSTTIRYQATGFGTNETEYLFEVDNLTYVQLESRFTPQFLLQLNETIYTSGKRSNTTGKLIWKVNPEIDTTIGEWAFWETKKNLTRKIRSEELSFTAVSNRAKNISGQSPARTSSDPGTNTTTEDHKIMASENSSAMVQVHSQGREAAVSHLTTLATISTSPQPPTTKPGPDNSTHNTPVYKLDISEATQAEQHHRRTDNDSTTSDTPPAMTAAGPPKAENTNTSKGTDLPDPATTTSPQNHSETAGNNNTHHQDTGEESASSGKLGLITNTIAGVAGLITGGRRTRREAIVNAQPKCNPNLHYWTTQDEGAAIGLAWIPYFGPAAEGIYTEGLMHNQDGLICGLRQLANETTQALQLFLRATTELRTFSILNRKAIDFLLQRWGGTCHILGPDCCIEPHDWTKNITDKIDQIIHDFVDKTLPDQGDNDNWWTGWRQWIPAGIGVTGVIIAVIALFCICKFVF

SEQ ID NO: 28 - protein, 677 aa, Reston ebolavirus
MGSGYQLLQLPRERFRKTSFLVWVIILFQRAISMPLGIVTNSTLKATEIDQLVCRDKLSSTSQLKSVGLNLEGNGIATDVPSATKRWGFRSGVPPKVVSYEAGEWAENCYNLEIKKSDGSECLPLPPDGVRGFPRCRYVHKVQGTGPCPGDLAFHKNGAFFLYDRLASTVIYRGTTFTEGVVAFLILSEPKKHFWKATPAHEPVNTTDDSTSYYMTLTLSYEMSNFGGKESNTLFKVDNHTYVQLDRPHTPQFLVQLNETLRRNNRLSNSTGRLTWTLDPKIEPDVGEWAFWETKKNFSQQLHGENLHFQILSTHTNNSSDQSPAGTVQGKISYHPPTNNSELVPTDSPPVVSVLTAGRTEEMSTQGLTNGETITGFTANPMTTTIAPSPTMTSEVDNNVPSEQPNNTASIEDSPPSASNETIDHSEMNPIQGSNNSAQSPQTKTTPAPTASPMTQDPQETANSSKLGTSPGSAAEPSQPGFTINTVSKVADSLSPTRKQKRSVRQNTANKCNPDLHYWTAVDEGAAVGLAWIPYFGPAAEGIYIEGVMHNQNGLICGLRQLANETTQALQLFLRATTELRTYSLLNRKAIDFLLQRWGGTCRILGPSCCIEPHDWTKNITDEINQIKHDFIDNPLPDHGDDLNLWTGWRQWIPAGIGIIGVIIAIIALLCICKILC

SEQ ID NO: 29 - protein, 676 aa, Tai Forest ebolavirus
MGASGILQLPRERFRKTSFFVWVIILFHKVFSIPLGVVHNNTLQVSDIDKFVCRDKLSSTSQLKSVGLNLEGNGVATDVPTATKRWGFRAGVPPKVVNCEAGEWAENCYNLAIKKVDGSECLPEAPEGVRDFPRCRYVHKVSGTGPCPGGLAFHKEGAFFLYDRLASTIIYRGTTFAEGVIAFLILPKARKDFFQSPPLHEPANMTTDPSSYYHTTTINYVVDNFGTNTTEFLFQVDHLTYVQLEARFTPQFLVLLNETIYSDNRRSNTTGKLIWKINPTVDTSMGEWAFWENKKNFTKTLSSEELSFVPVPETQNQVLDTTATVSPPISAHNHAAEDHKELVSEDSTPVVQMQNIKGKDTMPTTVTGVPTTTPSPFPINARNTDHTKSFIGLEGPQEDHSTTQPAKTTSQPTNSTESTTLNPTSEPSSRGTGPSSPTVPNTTESHAELGKTTPTTLPEQHTAASAIPRAVHPDELSGPGFLTNTIRGVTNLLTGSRRKRRDVTPNTQPKCNPNLHYWTALDEGAAIGLAWIPYFGPAAEGIYTEGIMENQNGLICGLRQLANETTQALQLFLRATTELRTFSILNRKAIDFLLQRWGGTCHILGPDCCIEPQDWTKNITDKIDQIIHDFVDNNLPNQNDGSNWWTGWKQWVPAGIGITGVIIAIIALLCICKFML

SEQ ID NO: 30 - protein, 364 aa, Zaire ebolavirus
MGVTGILQLPRDRFKRTSFFLWVIILFQRTFSIPLGVIHNSTLQVSDVDKLVCRDKLSSTNQLRSVGLNLEGNGVATDVPSATKRWGFRSGVPPKVVNYEAGEWAENCYNLEIKKPDGSECLPAAPDGIRGFPRCRYVHKVSGTGPCAGDFAFHKEGAFFLYDRLASTVIYRGTTFAEGVVAFLILPQAKKDFFSSHPLREPVNATEDPSSGYYSTTIRYQATGFGTNETEYLFEVDNLTYVQLESRFTPQFLLQLNETIYTSGKRSNTTGKLIWKVNPEIDTTIGEWAFWETKKTSLEKFAVKSCLSQLYQTEPKTSVVRVRRELLPTQGPTQQLKTTKSWLQKIPLQWFKCTVKEGKLQCRI

SEQ ID NO: 31 - protein, 19 aa, Artificial Sequence
  Synthetic peptide
IYYSGSTNYNPSLKSRVTI